European Patent Specification EP 3 659 586 B1, published June 21, 2023. Title: SOST Antibody Pharmaceutical Composition and Uses Thereof. Applicant: Jiangsu Hengrui Medicine Co., Ltd., Shanghai Hengrui Pharmaceutical Co., Ltd. The sequence listing filed with the application follows.

SEQUENCE LISTING (25 sequences)

SEQ ID NO: 1 - protein, 117 aa, murine
EVQLQQSGPELVKPGTSVKIPCQTSGYTFTDYNLDWLKQRPGESLEWIGDIDPNNGDILYNQKFRDKATLTVDTSSNTAYLELRSLTSEDTAVYYCARRWAYYFDYWGQGTTLTISS

SEQ ID NO: 2 - protein, 107 aa, murine
NIVMTQTPKLLFVSAGDRITITCKASQSVSNDVAWYQQKPGQSPKLLIYYTSNRFTGVPDRFTGSGYGTDFTLTINTVQAEDLAVYFCQQDYSSPVTFGAGTKLELK

SEQ ID NO: 3 - protein, 5 aa, murine
DYNLD

SEQ ID NO: 4 - protein, 17 aa, murine
DIDPNNGDILYNQKFRD

SEQ ID NO: 5 - protein, 8 aa, murine
RWAYYFDY

SEQ ID NO: 6 - protein, 11 aa, murine
KASQSVSNDVA

SEQ ID NO: 7 - protein, 7 aa, murine
YTSNRFT

SEQ ID NO: 8 - protein, 9 aa, murine
QQDYSSPVT

SEQ ID NO: 9 - protein, 17 aa, artificial sequence
  Mutant HCDR2
DIDPNDGDILYNQKFRD

SEQ ID NO: 10 - protein, 117 aa, artificial sequence
  Ab-5 heavy chain variable region
EVQLVQSGAEVKKPGASVKVSCKASGYTFTDYNLDWVRQAPGQGLEWMGDIDPNNGDILYNQKFRDRVTMTTDTSTSTAYMELRSLRSDDTAVYYCARRWAYYFDYWGQGTTVTVSS

SEQ ID NO: 11 - protein, 117 aa, artificial sequence
  Ab-9 heavy chain variable region
EVQLVQSGAEVKKPGASVKVSCKASGYTFTDYNLDWLRQAPGEGLEWIGDIDPNNGDILYNQKFRDRVTMTTDTSTSTAYMELRSLRSDDTAVYYCARRWAYYFDYWGQGTTVTVSS

SEQ ID NO: 12 - protein, 117 aa, artificial sequence
  Ab-10 heavy chain variable region
EVQLVQSGAEVKKPGASVKVSCKASGYTFTDYNLDWLRQAPGEGLEWIGDIDPNDGDILYNQKFRDRVTMTTDTSTSTAYMELRSLRSDDTAVYYCARRWAYYFDYWGQGTTVTVSS

SEQ ID NO: 13 - protein, 107 aa, artificial sequence
  Ab-5 light chain variable region
DIQMTQSPSSLSASVGDRVTITCKASQSVSNDVAWYQQKPGKAPKLLIYYTSNRFTGVPSRFSGSGSGTDFTLTISSLQPEDFATYYCQQDYSSPVTFGGGTKVEIK

SEQ ID NO: 14 - protein, 107 aa, artificial sequence
  Ab-9 light chain variable region
NIVMTQSPSSLSASVGDRVTITCKASQSVSNDVAWYQQKPGKSPKLLIYYTSNRFTGVPDRFSGSGSGTDFTLTISSLQPEDFATYFCQQDYSSPVTFGGGTKVEIK

SEQ ID NO: 15 - protein, 107 aa, artificial sequence
  Ab-10 light chain variable region
DIVMTQSPSSLSASVGDRVTITCKASQSVSNDVAWYQQKPGKSPKLLIYYTSNRFTGVPDRFSGSGSGTDFTLTISSLQPEDFATYFCQQDYSSPVTFGGGTKVEIK

SEQ ID NO: 16 - protein, 326 aa, Homo sapiens
ASTKGPSVFPLAPCSRSTSESTAALGCLVKDYFPEPVTVSWNSGALTSGVHTFPAVLQSSGLYSLSSVVTVPSSSLGTKTYTCNVDHKPSNTKVDKRVESKYGPPCPPCPAPEFLGGPSVFLFPPKPKDTLMISRTPEVTCVVVDVSQEDPEVQFNWYVDGVEVHNAKTKPREEQFNSTYRVVSVLTVLHQDWLNGKEYKCKVSNKGLPSSIEKTISKAKGQPREPQVYTLPPSQEEMTKNQVSLTCLVKGFYPSDIAVEWESNGQPENNYKTTPPVLDSDGSFFLYSRLTVDKSRWQEGNVFSCSVMHEALHNHYTQKSLSLSLG

SEQ ID NO: 17 - protein, 327 aa, Homo sapiens
ASTKGPSVFPLAPCSRSTSESTAALGCLVKDYFPEPVTVSWNSGALTSGVHTFPAVLQSSGLYSLSSVVTVPSSSLGTKTYTCNVDHKPSNTKVDKRVESKYGPPCPPCPAPEFLGGPSVFLFPPKPKDTLMISRTPEVTCVVVDVSQEDPEVQFNWYVDGVEVHNAKTKPREEQFNSTYRVVSVLTVLHQDWLNGKEYKCKVSNKGLPSSIEKTISKAKGQPREPQVYTLPPSQEEMTKNQVSLTCLVKGFYPSDIAVEWESNGQPENNYKTTPPVLDSDGSFFLYSRLTVDKSRWQEGNVFSCSVMHEALHNHYTQKSLSLSLGK

SEQ ID NO: 18 - protein, 330 aa, Homo sapiens [sequence omitted]

SEQ ID NO: 19 - protein, 107 aa, Homo sapiens [sequence omitted]

SEQ ID NO: 20 - protein, 447 aa, artificial sequence
  humanized antibody Ab-10 heavy chain
EVQLVQSGAEVKKPGASVKVSCKASGYTFTDYNLDWVRQAPGQGLEWMGDIDPNNGDILYNQKFRDRVTMTTDTSTSTAYMELRSLRSDDTAVYYCARRWAYYFDYWGQGTTVTVSSASTKGPSVFPLAPSSKSTSGGTAALGCLVKDYFPEPVTVSWNSGALTSGVHTFPAVLQSSGLYSLSSVVTVPSSSLGTQTYICNVNHKPSNTKVDKKVEPKSCDKTHTCPPCPAPELLGGPSVFLFPPKPKDTLMISRTPEVTCVVVDVSHEDPEVKFNWYVDGVEVHNAKTKPREEQYNSTYRVVSVLTVLHQDWLNGKEYKCKVSNKALPAPIEKTISKAKGQPREPQVYTLPPSRDELTKNQVSLTCLVKGFYPSDIAVEWESNGQPENNYKTTPPVLDSDGSFFLYSKLTVDKSRWQQGNVFSCSVMHEALHNHYTQKSLSLSPGK

SEQ ID NO: 21 - protein, 444 aa, artificial sequence
  humanized antibody Ab-9 heavy chain
EVQLVQSGAEVKKPGASVKVSCKASGYTFTDYNLDWLRQAPGEGLEWIGDIDPNNGDILYNQKFRDRVTMTTDTSTSTAYMELRSLRSDDTAVYYCARRWAYYFDYWGQGTTVTVSSASTKGPSVFPLAPCSRSTSESTAALGCLVKDYFPEPVTVSWNSGALTSGVHTFPAVLQSSGLYSLSSVVTVPSSSLGTKTYTCNVDHKPSNTKVDKRVESKYGPPCPPCPAPEFLGGPSVFLFPPKPKDTLMISRTPEVTCVVVDVSQEDPEVQFNWYVDGVEVHNAKTKPREEQFNSTYRVVSVLTVLHQDWLNGKEYKCKVSNKGLPSSIEKTISKAKGQPREPQVYTLPPSQEEMTKNQVSLTCLVKGFYPSDIAVEWESNGQPENNYKTTPPVLDSDGSFFLYSRLTVDKSRWQEGNVFSCSVMHEALHNHYTQKSLSLSLGK

SEQ ID NO: 22 - protein, 443 aa, artificial sequence
  humanized antibody Ab-5 heavy chain
EVQLVQSGAEVKKPGASVKVSCKASGYTFTDYNLDWLRQAPGEGLEWIGDIDPNDGDILYNQKFRDRVTMTTDTSTSTAYMELRSLRSDDTAVYYCARRWAYYFDYWGQGTTVTVSSASTKGPSVFPLAPCSRSTSESTAALGCLVKDYFPEPVTVSWNSGALTSGVHTFPAVLQSSGLYSLSSVVTVPSSSLGTKTYTCNVDHKPSNTKVDKRVESKYGPPCPPCPAPEFLGGPSVFLFPPKPKDTLMISRTPEVTCVVVDVSQEDPEVQFNWYVDGVEVHNAKTKPREEQFNSTYRVVSVLTVLHQDWLNGKEYKCKVSNKGLPSSIEKTISKAKGQPREPQVYTLPPSQEEMTKNQVSLTCLVKGFYPSDIAVEWESNGQPENNYKTTPPVLDSDGSFFLYSRLTVDKSRWQEGNVFSCSVMHEALHNHYTQKSLSLSLG

SEQ ID NO: 23 - protein, 214 aa, artificial sequence
  humanized antibody Ab-10 light chain
DIQMTQSPSSLSASVGDRVTITCKASQSVSNDVAWYQQKPGKAPKLLIYYTSNRFTGVPSRFSGSGSGTDFTLTISSLQPEDFATYYCQQDYSSPVTFGGGTKVEIKRTVAAPSVFIFPPSDEQLKSGTASVVCLLNNFYPREAKVQWKVDNALQSGNSQESVTEQDSKDSTYSLSSTLTLSKADYEKHKVYACEVTHQGLSSPVTKSFNRGEC

SEQ ID NO: 24 - protein, 214 aa, artificial sequence
  humanized antibody Ab-9 light chain
NIVMTQSPSSLSASVGDRVTITCKASQSVSNDVAWYQQKPGKSPKLLIYYTSNRFTGVPDRFSGSGSGTDFTLTISSLQPEDFATYFCQQDYSSPVTFGGGTKVEIKRTVAAPSVFIFPPSDEQLKSGTASVVCLLNNFYPREAKVQWKVDNALQSGNSQESVTEQDSKDSTYSLSSTLTLSKADYEKHKVYACEVTHQGLSSPVTKSFNRGEC

SEQ ID NO: 25 - protein, 214 aa, artificial sequence
  humanized antibody Ab-5 light chain
DIVMTQSPSSLSASVGDRVTITCKASQSVSNDVAWYQQKPGKSPKLLIYYTSNRFTGVPDRFSGSGSGTDFTLTISSLQPEDFATYFCQQDYSSPVTFGGGTKVEIKRTVAAPSVFIFPPSDEQLKSGTASVVCLLNNFYPREAKVQWKVDNALQSGNSQESVTEQDSKDSTYSLSSTLTLSKADYEKHKVYACEVTHQGLSSPVTKSFNRGEC